European Patent Application EP 4 311 860 A1, published January 31, 2024. Title: MÉTHODE D'ÉVALUATION IN VITRO DE L'ACTIVITÉ PHOTOPROTECTRICE D'UN ACTIF. Applicant: PIERRE FABRE DERMOCOSMETIQUE. The sequence listing filed with the application follows.

SEQUENCE LISTING (6 sequences)

SEQ ID NO: 1 - DNA, 15 bp, synthetic construct
  source 1..15: mol_type = other DNA
catcttacattttac

SEQ ID NO: 2-3 - skipped (2 entries)

SEQ ID NO: 4 - DNA, 10 bp, synthetic construct
  source 1..10: mol_type = other DNA
tattgttgca

SEQ ID NO: 5 - DNA, 15 bp, synthetic construct
  source 1..15: mol_type = other DNA
cattgtattgttgca

SEQ ID NO: 6 - DNA, 21 bp, synthetic construct
  source 1..21: mol_type = other DNA
attgtattgtattgattgcaa